European Patent Application EP 4 112 643 A1, published January 4, 2023. Title: Monoclonal antibody specifically binding to TIM-3 and uses thereof. Applicant: NATIONAL CANCER CENTER. The sequence listing filed with the application follows.

SEQUENCE LISTING (18 sequences)

SEQ ID NO: 1 - protein, 9 aa, Artificial
  heavy chain CDR1_amino acid
SIFSNGYMT

SEQ ID NO: 2 - protein, 9 aa, Artificial
  heavy chain CDR2_amino acid
SINSRGVTN

SEQ ID NO: 3 - protein, 11 aa, Artificial
  heavy chain CDR3_amino acid
AALLPHEIRKY

SEQ ID NO: 4 - protein, 17 aa, Artificial
  light chain CDR1_amino acid
KSSQSVFYNSNNKNYLG

SEQ ID NO: 5 - protein, 7 aa, Artificial
  light chain CDR2_amino acid
WASTRES

SEQ ID NO: 6 - protein, 10 aa, Artificial
  light chain CDR3_amino acid
CQQYYSTPRT

SEQ ID NO: 7 - protein, 117 aa, Artificial
  heavy chain variable region_amino acid
EVQLVESGGGLVQPGGSLRLSCAASGSIFSNGYMTWYRQAPGKGLELVSSINSRGVTNYADSVKGRFTISRDNSKNTLYLQMNSLRAEDTAVYYCAALLPHEIRKYWGQGTQVTVSS

SEQ ID NO: 8 - protein, 116 aa, Artificial
  light chain variable region_amino acid
VDDIQMTQSPDSLAVSLGERATINCKSSQSVFYNSNNKNYLGWYQKKPGQPPKLLIFWASTRESGVPDRFSGSGSGTDFTLTISSLQAEDVAVYYCQQYYSTPRTLGGGTKVDIKR

SEQ ID NO: 9 - protein, 13 aa, Artificial
  linker_amino acid
GGGSHGGGSGGGS

SEQ ID NO: 10 - DNA, 27 bp, Artificial
  heavy chain CDR1_nucleotide
tcactgcgtctgagctgcgcggccagc

SEQ ID NO: 11 - DNA, 27 bp, Artificial
  heavy chain CDR2_nucleotide
gcgcccgggaaaggtctggaattggtg

SEQ ID NO: 12 - DNA, 33 bp, Artificial
  heavy chain CDR3_nucleotide
gccgccctgcttcctcatgagattcggaagtat

SEQ ID NO: 13 - DNA, 51 bp, Artificial
  light chain CDR1_nucleotide
aagtccagccagagtgttttttacaactccaacaataagaactacttaggt

SEQ ID NO: 14 - DNA, 21 bp, Artificial
  light chain CDR2_nucleotide
tgggcatctacccgggaatcc

SEQ ID NO: 15 - DNA, 30 bp, Artificial
  light chain CDR3_nucleotide
tgtcagcaatattatagcactcctcgcact

SEQ ID NO: 16 - DNA, 351 bp, Artificial
  heavy chain variable region_nucleotide
gaagtgcagctggtggaatcgggtggtggtctggttcaaccgggcggctcactgcgtctgagctgcgcggccagcggtagtatctttagtaatggttatatgacttggtatcgtcaggcgcccgggaaaggtctggaattggtgtcgtcgattaattcgaggggagtgaccaattatgcagactctgttaaaggccgttttaccatcagccgcgataactctaaaaatacgctgtatctgcaaatgaactctctgcgcgcggaagatacggcagtgtattactgcgccgccctgcttcctcatgagattcggaagtattggggtcagggtacccaagtgacggttagctct

SEQ ID NO: 17 - DNA, 348 bp, Artificial
  light chain variable region_nucleotide
gtcgacgacatccagatgacccagtctccagactccctggctgtgtctctgggcgagagggccaccatcaactgcaagtccagccagagtgttttttacaactccaacaataagaactacttaggttggtaccagaagaaaccaggacagcctcctaagctgctcattttctgggcatctacccgggaatccggggtccctgaccgattcagtggcagcgggtctgggacagatttcactctcaccatcagcagcctgcaggctgaagatgtggcagtttattactgtcagcaatattatagcactcctcgcactctcggcggagggaccaaagtggatatcaaacgt

SEQ ID NO: 18 - DNA, 39 bp, Artificial
  linker_nucleotide
ggtggcggttcacatggtggcggcagcggaggtggatcc